European Patent Application EP 4 631 535 A1, published October 15, 2025. Title: Compounds for use as bone replacement and/or bone rebuilding material. Applicant: novaxomx GmbH. The sequence listing filed with the application follows.

SEQUENCE LISTING (20 sequences)

SEQ ID NO: 1 - DNA, 20 bp, Homo sapiens
  source 1..20: mol_type = other DNA
cagacaagtcccacacagca

SEQ ID NO: 2 - DNA, 20 bp, Homo sapiens
  source 1..20: mol_type = other DNA
cttggcatctgtgaggtcag

SEQ ID NO: 3 - DNA, 20 bp, Homo sapiens
  source 1..20: mol_type = other DNA
ccgagtgtgtgagtgtgagg

SEQ ID NO: 4 - DNA, 20 bp, Homo sapiens
  source 1..20: mol_type = other DNA
tgtgtttcgctctggggttc

SEQ ID NO: 5 - DNA, 20 bp, Homo sapiens
  source 1..20: mol_type = other DNA
tgcagctcaacaaggatacg

SEQ ID NO: 6 - DNA, 20 bp, Homo sapiens
  source 1..20: mol_type = other DNA
gtgcagttggtccaaggttt

SEQ ID NO: 7 - DNA, 20 bp, Homo sapiens
  source 1..20: mol_type = other DNA
gcagaaggaactgcaacaca

SEQ ID NO: 8 - DNA, 20 bp, Homo sapiens
  source 1..20: mol_type = other DNA
gatggtgaggtgtgcaaatg

SEQ ID NO: 9 - DNA, 18 bp, Homo sapiens
  source 1..18: mol_type = other DNA
gccgggaatgatgagaac

SEQ ID NO: 10 - DNA, 19 bp, Homo sapiens
  source 1..19: mol_type = other DNA
ggaccgtccactgtcactt

SEQ ID NO: 11 - DNA, 20 bp, Homo sapiens
  source 1..20: mol_type = other DNA
ccaatgccaaagagatcgcc

SEQ ID NO: 12 - DNA, 22 bp, Homo sapiens
  source 1..22: mol_type = other DNA
tctgtgcagagacgttgccaag

SEQ ID NO: 13 - DNA, 20 bp, Homo sapiens
  source 1..20: mol_type = other DNA
gagagcatgaccgatggatt

SEQ ID NO: 14 - DNA, 20 bp, Homo sapiens
  source 1..20: mol_type = other DNA
tgagctcgatctcgttggat

SEQ ID NO: 15 - DNA, 20 bp, Homo sapiens
  source 1..20: mol_type = other DNA
acggcatggatctcaaagac

SEQ ID NO: 16 - DNA, 20 bp, Homo sapiens
  source 1..20: mol_type = other DNA
gtgggtgaggagcacgtagt

SEQ ID NO: 17 - DNA, 20 bp, Homo sapiens
  source 1..20: mol_type = other DNA
tgtgaacggatttggccgta

SEQ ID NO: 18 - DNA, 20 bp, Homo sapiens
  source 1..20: mol_type = other DNA
actgtgccgttgaatttgcc

SEQ ID NO: 19 - DNA, 19 bp, Homo sapiens
  source 1..19: mol_type = other DNA
gaagttcggccagggttcc

SEQ ID NO: 20 - DNA, 20 bp, Homo sapiens
  source 1..20: mol_type = other DNA
gaagcctatgtccttcgcgt